European Patent Specification EP 3 681 903 B1, published July 19, 2023. Title: COMPOSITIONS AND METHODS FOR TREATING CANCER WITH ANTI-CD19 IMMUNOTHERAPY. Applicant: Lentigen Technology, Inc. The sequence listing filed with the application follows.

SEQUENCE LISTING (51 sequences)

SEQ ID NO: 1 - DNA, 741 bp, Artificial Sequence
  CD19-reactive ScFv1 binding domain (LTG2050)
gaggtccagctggtacagtctggagctgaggtgaagaagcctggggcctcagtgaaggtctcctgcaaggcttctggatacaccttcaccagctactatatgcactgggtgcgacaggcccctggacaagggcttgagtggatgggaataatcaaccctagtggtggtagcacaagctacgcacagaagttccagggcagagtcaccatgaccagggacacgtccacgagcacagtctacatggagctgagcagcctgagatctgaggacacggccgtgtattactgtgcgagatcggatcggggaattaccgccacggacgcttttgatatctggggccaagggacaatggtcaccgtctcttcaggaggtggcgggtctggtggaggcggtagcggtggtggcggatcccagtctgtgctgactcagccaccctcggtgtcagtggccccagggcagacggccaagattacctgtgggggaagtgacattggaaataaaaatgtccactggtaccagcagaagccaggccaggcccctgtcctggtcgtctatgatgattacgaccggccctcagggatccctgagcgattctctggctccaactctggggacgcggccaccctgacgatcagcacggtcgaagtcggggatgaggccgactatttctgtcaggtgtgggacagtagtggtgatccttattgggtgttcggcggagggacccagctcaccgttttaggt

SEQ ID NO: 2 - protein, 247 aa, Artificial Sequence
  CD19-reactive ScFv1 binding domain (LTG2050)
EVQLVQSGAEVKKPGASVKVSCKASGYTFTSYYMHWVRQAPGQGLEWMGIINPSGGSTSYAQKFQGRVTMTRDTSTSTVYMELSSLRSEDTAVYYCARSDRGITATDAFDIWGQGTMVTVSSGGGGSGGGGSGGGGSQSVLTQPPSVSVAPGQTAKITCGGSDIGNKNVHWYQQKPGQAPVLVVYDDYDRPSGIPERFSGSNSGDAATLTISTVEVGDEADYFCQVWDSSGDPYWVFGGGTQLTVLG

SEQ ID NO: 3 - DNA, 741 bp, Artificial Sequence
  CD19-reactive ScFv2 binding domain (LTG2065)
gaggtccagctggtacagtctggagctgaggtgaagaagcctggggcctcagtgaaggtctcctgcaaggcttctggatacaccttcaccagctactatatgcactgggtgcgacaggcccctggacaagggcttgagtggatgggattaatcaaccctagtggtggtagcacaagctacgcacagaagttccagggcagagtcaccatgaccagggacacgtccacgagcacagtctacatggagctgagcagcctgagatctgaggacacggccgtgtattactgtgcgagatcggatcggggaattaccgccacggacgcttttgatatctggggccaagggacaatggtcaccgtctcttcaggcggaggaggctccgggggaggaggttccgggggcgggggttcccagtctgtgctgactcagccaccctcggtgtcagtggccccagggcggatggccaagattacctgtgggggaagtgacattggaaataaaaatgtccactggtatcagcagaagccaggccaggcccctgtcctggttgtctatgatgattacgaccggccctcagggatccctgagcgattctctggctccaactctggggacgcggccaccctgacgatcagcacggtcgaagtcggggatgaggccgactatttctgtcaggtgtgggacggtagtggtgatccttattggatgttcggcggagggacccagctcaccgttttaggt

SEQ ID NO: 4 - protein, 247 aa, Artificial Sequence
  CD19-reactive ScFv2 binding domain (LTG2065)
EVQLVQSGAEVKKPGASVKVSCKASGYTFTSYYMHWVRQAPGQGLEWMGLINPSGGSTSYAQKFQGRVTMTRDTSTSTVYMELSSLRSEDTAVYYCARSDRGITATDAFDIWGQGTMVTVSSGGGGSGGGGSGGGGSQSVLTQPPSVSVAPGRMAKITCGGSDIGNKNVHWYQQKPGQAPVLVVYDDYDRPSGIPERFSGSNSGDAATLTISTVEVGDEADYFCQVWDGSGDPYWMFGGGTQLTVLG

SEQ ID NO: 5 - DNA, 741 bp, Artificial Sequence
  CD19-reactive ScFv3 binding domain (LTG2066)
gaggtccagctggtacagtctggagctgaggtgaagaagcctggggcctcagtgaaggtctcctgcaaggcttccggatacaccttcaccagctactacatgcactgggtgcgacaggcccctggacaagggtttgagtggatgggattaatcaaccctagtggtagtagcacaagctacgcacagaagttccagggcagagtcaccatgaccagggacacgtccacgagcacagtctacatggagctgagcaacctgagatctgaggacacggccgtgtattactgtgcgagatcggatcggggaattaccgccacggacgcttttgatatctggggccaagggacaatggtcaccgtctcttcaggcggaggaggctccgggggaggaggttccgggggcgggggttcccagtctgtgctgactcagccaccctcggtgccagtggccccagggcagacggccaagattatctgtgggggaagtgacattggaaataaaaatgtccactggtaccagcagaagccaggccaggcccctgtcctggtcgtctatgatgactacgaccggccctcagggatccctgagcgattctctggctccaactctggggacgcggccaccctgacgatcagcacggttgaagtcggggatgaggccgactatttctgtcaggtgtgggacggtagtggtgatccttattgggtgttcggcggagggacccagctcaccgtcttaggt

SEQ ID NO: 6 - protein, 247 aa, Artificial Sequence
  CD19-reactive ScFv3 binding domain (LTG2066)
EVQLVQSGAEVKKPGASVKVSCKASGYTFTSYYMHWVRQAPGQGFEWMGLINPSGSSTSYAQKFQGRVTMTRDTSTSTVYMELSNLRSEDTAVYYCARSDRGITATDAFDIWGQGTMVTVSSGGGGSGGGGSGGGGSQSVLTQPPSVPVAPGQTAKIICGGSDIGNKNVHWYQQKPGQAPVLVVYDDYDRPSGIPERFSGSNSGDAATLTISTVEVGDEADYFCQVWDGSGDPYWVFGGGTQLTVLG

SEQ ID NO: 7 - DNA, 741 bp, Artificial Sequence
  CD19-reactive ScFv4 binding domain (LTG2067)
gaggtccagctggtacagtctggagctgaggtgaacaagcctggtgcctcagtgaaggtctcctgcaaggcttctggatacaccttcaccagctactatatgcactgggtgcgacaggcccctggacaagggcttgagtggatgggaatgatcaaccctagtggtggtagcacaagctacgcacagaagttccagggcagagtcaccatgaccagggacacgtccacgagcacagtctacatggagctgagcagcctgagatctgaggacacggccgtgtattactgtgcgagatcggatcggggaattacctccacggacgcttttgatatctggggccaagggacaatggtcaccgtctcttcaggcggaggaggctccgggggaggaggttccgggggcgggggttcccagtctgtgctgactcagccaccctcggtgtcattggccccagggcagacggccaagattacctgtgggggaagtgacattggaaataaaaatgtccactggtaccagcagaagccaggccaggcccctgtcctagtcgtctatgatgattacaaccggccctcagggatccctgagcgattctctggctccaactctggggactcagccaccctgacgatcagcacggtcgaagtcggggatgaggccgactatttctgtcaggtgtgggacggtagtggtgatccttattgggtgttcggcggagggacccagctcaccgttttaggt

SEQ ID NO: 8 - protein, 247 aa, Artificial Sequence
  CD19-reactive ScFv4 binding domain (LTG2067)
EVQLVQSGAEVNKPGASVKVSCKASGYTFTSYYMHWVRQAPGQGLEWMGMINPSGGSTSYAQKFQGRVTMTRDTSTSTVYMELSSLRSEDTAVYYCARSDRGITSTDAFDIWGQGTMVTVSSGGGGSGGGGSGGGGSQSVLTQPPSVSLAPGQTAKITCGGSDIGNKNVHWYQQKPGQAPVLVVYDDYNRPSGIPERFSGSNSGDSATLTISTVEVGDEADYFCQVWDGSGDPYWVFGGGTQLTVLG

SEQ ID NO: 9 - DNA, 741 bp, Artificial Sequence
  CD19-reactive ScFv5 binding domain (LTG2068)
gaggtccagctggtacagtctggagctgaggtgaagaagcctggggcctcagtgaaggtctcctgcaaggcatctggatacaccttcaccggctactatatgcactgggtgcggcaggcccctggacaagggcttgagtggataggattaatcaaccctagtggtggtagcacaagctacgaacagaagttccagggcagagtcgccatgaccagggacacgtcaacgagcacagtctacatggagctgagcagcctgagatctgaggacacggccgtgtattactgtgcgagatcggatcggggaattaccgccacggacgcttttgatatctggggccaagggacaatggtcaccgtctcttcaggcggaggaggctccgggggaggaggttccgggggcgggggttcccagtctgtgctgactcagccaccctcggtgtcagtggccccagggcagacggccaagattacctgtgggggaagtgacattggagataaaaatgtccactggtaccagcagaagccaggccaggcccctgtcctggtcgtctatgatgattacgaccggccctcagggatccctgagcgattctctggctccaactctggggacgcggccaccctgacgatcagcacggtcgaagtcggggatgaggccgactatttctgtcaggtgtgggacggtattggtgatccctattgggtgttcggcggagggacccagctcaccgttttaggt

SEQ ID NO: 10 - protein, 247 aa, Artificial Sequence
  CD19-reactive ScFv5 binding domain (LTG2068)
EVQLVQSGAEVKKPGASVKVSCKASGYTFTGYYMHWVRQAPGQGLEWIGLINPSGGSTSYEQKFQGRVAMTRDTSTSTVYMELSSLRSEDTAVYYCARSDRGITATDAFDIWGQGTMVTVSSGGGGSGGGGSGGGGSQSVLTQPPSVSVAPGQTAKITCGGSDIGDKNVHWYQQKPGQAPVLVVYDDYDRPSGIPERFSGSNSGDAATLTISTVEVGDEADYFCQVWDGIGDPYWVFGGGTQLTVLG

SEQ ID NO: 11 - DNA, 741 bp, Artificial Sequence
  CD19-reactive ScFv6 binding domain (LTG2069)
gaggtccagctagtacagtctggagctgaggtgaagaagcctggggcctcagtgaaggtctcctgcaaggcttctggatacaccttcaccagctactatatgcactgggtgcgacaggcccctggacaagggcttgagtggatgggaatgatcaaccctagtggtggtagcacaagctacgcacagaagttccagggcagagtcaccatgaccagggacacgtccacgagcacagtctacatggagctgagcagcctgagatctgaggacacggccgtgtattactgtgcgagatcggatcggggaattaccgccacggacgcttttgatatctggggccaagggacaatggtcaccgtctcttcaggcggaggaggctccgggggaggaggttccgggggcgggggttcccagtctgtgctgactcagccaccctcggtgtcagtggccccagggcagacggccaagattacctgtgggggaagtgacattggaaataaaaatgcccactggtaccagcagaagccaggccaggcccctgtcctggtcgtctatgatgattacgaccggccctcagggatctctgagcgattctctggctccaactctggggacgcggccaccctgacgatcagcacggtcgaagtcggggatgaggccgactatttctgtcaggtgtgggacggtagtggtgatcctttttgggtgttcggcggagggacccagctcaccgttttaggt

SEQ ID NO: 12 - protein, 247 aa, Artificial Sequence
  CD19-reactive ScFv6 binding domain (LTG2069)
EVQLVQSGAEVKKPGASVKVSCKASGYTFTSYYMHWVRQAPGQGLEWMGMINPSGGSTSYAQKFQGRVTMTRDTSTSTVYMELSSLRSEDTAVYYCARSDRGITATDAFDIWGQGTMVTVSSGGGGSGGGGSGGGGSQSVLTQPPSVSVAPGQTAKITCGGSDIGNKNAHWYQQKPGQAPVLVVYDDYDRPSGISERFSGSNSGDAATLTISTVEVGDEADYFCQVWDGSGDPFWVFGGGTQLTVLG

SEQ ID NO: 13 - DNA, 741 bp, Artificial Sequence
  CD19-reactive ScFv7 binding domain (LTG2070)
gaggtccagctggtacagtctggagctgaggtgaagaggcctggggcctcagtgaaggtctcctgcaaggcttctggatacaccttcaccagctactatatgcactgggtgcgacaggcccctggacgagggcttgagtggatgggattaatcaaccctagtggtggtagcacaagctacgcacaggagttccagggcagagtcaccatgaccagggacatgtccacgagcacagtctacatggagctgagcagcctgagatctgaggacacggccgtgtattactgtgcgagatcggatcggggaattagcgccacggacgcttttgatatctggggccaagggacaatggtcaccgtctcttcaggcggaggaggctccgggggaggaggttccgggggcgggggttcccagtctgtgctgactcagccaccctcggtgtcagtggccccagggcagatggccaagattacctgtgggggaagtgacattggaaataaaaatgtccactggtaccagcagaagccaggccaggcccctgtcctggtcgtctatgatgattacaaccggccctcagggatccctgagcgattctctggctccaactctggggacgcggccaccctgacgatcagcacggtcgaagtcggggatgaggccgactatttctgtcaggtatgggacggtagtggtgatccttattgggtgttcggcggagggacccagctcaccgatttaggt

SEQ ID NO: 14 - protein, 247 aa, Artificial Sequence
  CD19-reactive ScFv7 binding domain (LTG2070)
EVQLVQSGAEVKRPGASVKVSCKASGYTFTSYYMHWVRQAPGRGLEWMGLINPSGGSTSYAQEFQGRVTMTRDMSTSTVYMELSSLRSEDTAVYYCARSDRGISATDAFDIWGQGTMVTVSSGGGGSGGGGSGGGGSQSVLTQPPSVSVAPGQMAKITCGGSDIGNKNVHWYQQKPGQAPVLVVYDDYNRPSGIPERFSGSNSGDAATLTISTVEVGDEADYFCQVWDGSGDPYWVFGGGTQLTDLG

SEQ ID NO: 15 - DNA, 741 bp, Artificial Sequence
  CD19-reactive ScFv8 binding domain (LTG2071)
gaggtccagctggtacagtctggagctgaggtgaagaggcctggggcctcagtgaaggtctcctgcaaggcttctggatacaccttcaccagctactatatgcactgggtgcgacaggcccctggacaagggcttgtgtggatgggattaatcaaccctagtggtggcagcacaagctacgcacagaagttccagggcagagtcaccatgaccagggacacgtccacgagcacagtctacatggagctgagcagcctgagatctgaggacacggccgtgtattactgtgcgagatcggatcggggaattaccgccacggacgcttttgatatctggggccaagggacaatggtcaccgtctcttcaggcggaggaggctccgggggaggaggttccgggggcgggggttcccagtctgtgctgactcagccaccctcggtctcagtggccccagggcagacggccaagactacctgtgggggaagtgacattggaaataaaaatgtccactggtaccagcagaagccaggccaggcccctgtcctggtcgtctatgatgattacgaccggccctcagggatccctgagcgattctctggctccaactctggggacgcggccaccctgacgatcagcacggtcgaagtcggggatgaggccgactatgtctgtcaggtgtgggacggtagtggtgatccttattgggtgttcggcggagggacccagctcaccgttttaggt

SEQ ID NO: 16 - protein, 247 aa, Artificial Sequence
  CD19-reactive ScFv8 binding domain (LTG2071)
EVQLVQSGAEVKRPGASVKVSCKASGYTFTSYYMHWVRQAPGQGLVWMGLINPSGGSTSYAQKFQGRVTMTRDTSTSTVYMELSSLRSEDTAVYYCARSDRGITATDAFDIWGQGTMVTVSSGGGGSGGGGSGGGGSQSVLTQPPSVSVAPGQTAKTTCGGSDIGNKNVHWYQQKPGQAPVLVVYDDYDRPSGIPERFSGSNSGDAATLTISTVEVGDEADYVCQVWDGSGDPYWVFGGGTQLTVLG

SEQ ID NO: 17 - DNA, 66 bp, Artificial Sequence
  leader/signal peptide sequence (LP)
atgctgctgctggtgaccagcctgctgctgtgcgaactgccgcatccggcgtttctgctgattccg

SEQ ID NO: 18 - protein, 22 aa, Artificial Sequence
  leader/signal peptide sequence (LP)
MLLLVTSLLLCELPHPAFLLIP

SEQ ID NO: 19 - DNA, 1485 bp, Artificial Sequence
  LTG2050_(LP-M19217-CD8 TM-41BB-CD3 zeta)
atgcttctcctggtcacctccctgctcctctgcgaactgcctcaccctgccttccttctgattcctgaggtccagctggtacagtctggagctgaggtgaagaagcctggggcctcagtgaaggtctcctgcaaggcttctggatacaccttcaccagctactatatgcactgggtgcgacaggcccctggacaagggcttgagtggatgggaataatcaaccctagtggtggtagcacaagctacgcacagaagttccagggcagagtcaccatgaccagggacacgtccacgagcacagtctacatggagctgagcagcctgagatctgaggacacggccgtgtattactgtgcgagatcggatcggggaattaccgccacggacgcttttgatatctggggccaagggacaatggtcaccgtctcttcaggaggtggcgggtctggtggaggcggtagcggtggtggcggatcccagtctgtgctgactcagccaccctcggtgtcagtggccccagggcagacggccaagattacctgtgggggaagtgacattggaaataaaaatgtccactggtaccagcagaagccaggccaggcccctgtcctggtcgtctatgatgattacgaccggccctcagggatccctgagcgattctctggctccaactctggggacgcggccaccctgacgatcagcacggtcgaagtcggggatgaggccgactatttctgtcaggtgtgggacagtagtggtgatccttattgggtgttcggcggagggacccagctcaccgttttaggtgcggccgcaactaccacccctgcccctcggccgccgactccggccccaaccatcgcaagccaacccctctccttgcgccccgaagcttgccgcccggccgcgggtggagccgtgcatacccgggggctggactttgcctgcgatatctacatttgggccccgctggccggcacttgcggcgtgctcctgctgtcgctggtcatcaccctttactgcaagaggggccggaagaagctgctttacatcttcaagcagccgttcatgcggcccgtgcagacgactcaggaagaggacggatgctcgtgcagattccctgaggaggaagaggggggatgcgaactgcgcgtcaagttctcacggtccgccgacgcccccgcatatcaacagggccagaatcagctctacaacgagctgaacctgggaaggagagaggagtacgacgtgctggacaagcgacgcggacgcgacccggagatgggggggaaaccacggcggaaaaaccctcaggaaggactgtacaacgaactccagaaagacaagatggcggaagcctactcagaaatcgggatgaagggagagcggaggaggggaaagggtcacgacgggctgtaccagggactgagcaccgccactaaggatacctacgatgccttgcatatgcaagcactcccaccccgg

SEQ ID NO: 20 - protein, 495 aa, Artificial Sequence
  LTG2050_(LP-M19217-CD8 TM-41BB-CD3zeta)
MLLLVTSLLLCELPHPAFLLIPEVQLVQSGAEVKKPGASVKVSCKASGYTFTSYYMHWVRQAPGQGLEWMGIINPSGGSTSYAQKFQGRVTMTRDTSTSTVYMELSSLRSEDTAVYYCARSDRGITATDAFDIWGQGTMVTVSSGGGGSGGGGSGGGGSQSVLTQPPSVSVAPGQTAKITCGGSDIGNKNVHWYQQKPGQAPVLVVYDDYDRPSGIPERFSGSNSGDAATLTISTVEVGDEADYFCQVWDSSGDPYWVFGGGTQLTVLGAAATTTPAPRPPTPAPTIASQPLSLRPEACRPAAGGAVHTRGLDFACDIYIWAPLAGTCGVLLLSLVITLYCKRGRKKLLYIFKQPFMRPVQTTQEEDGCSCRFPEEEEGGCELRVKFSRSADAPAYQQGQNQLYNELNLGRREEYDVLDKRRGRDPEMGGKPRRKNPQEGLYNELQKDKMAEAYSEIGMKGERRRGKGHDGLYQGLSTATKDTYDALHMQALPPR

SEQ ID NO: 21 - DNA, 1485 bp, Artificial Sequence
  LTG2065 (LP-M19217-1-CD8 TM-41BB-CD3 zeta)
atgctgctgctggtgaccagcctgctgctgtgcgaactgccgcatccggcgtttctgctgattccggaggtccagctggtacagtctggagctgaggtgaagaagcctggggcctcagtgaaggtctcctgcaaggcttctggatacaccttcaccagctactatatgcactgggtgcgacaggcccctggacaagggcttgagtggatgggattaatcaaccctagtggtggtagcacaagctacgcacagaagttccagggcagagtcaccatgaccagggacacgtccacgagcacagtctacatggagctgagcagcctgagatctgaggacacggccgtgtattactgtgcgagatcggatcggggaattaccgccacggacgcttttgatatctggggccaagggacaatggtcaccgtctcttcaggcggaggaggctccgggggaggaggttccgggggcgggggttcccagtctgtgctgactcagccaccctcggtgtcagtggccccagggcggatggccaagattacctgtgggggaagtgacattggaaataaaaatgtccactggtatcagcagaagccaggccaggcccctgtcctggttgtctatgatgattacgaccggccctcagggatccctgagcgattctctggctccaactctggggacgcggccaccctgacgatcagcacggtcgaagtcggggatgaggccgactatttctgtcaggtgtgggacggtagtggtgatccttattggatgttcggcggagggacccagctcaccgttttaggtgcggccgcaactaccacccctgcccctcggccgccgactccggccccaaccatcgcaagccaacccctctccttgcgccccgaagcttgccgcccggccgcgggtggagccgtgcatacccgggggctggactttgcctgcgatatctacatttgggccccgctggccggcacttgcggcgtgctcctgctgtcgctggtcatcaccctttactgcaagaggggccggaagaagctgctttacatcttcaagcagccgttcatgcggcccgtgcagacgactcaggaagaggacggatgctcgtgcagattccctgaggaggaagaggggggatgcgaactgcgcgtcaagttctcacggtccgccgacgcccccgcatatcaacagggccagaatcagctctacaacgagctgaacctgggaaggagagaggagtacgacgtgctggacaagcgacgcggacgcgacccggagatgggggggaaaccacggcggaaaaaccctcaggaaggactgtacaacgaactccagaaagacaagatggcggaagcctactcagaaatcgggatgaagggagagcggaggaggggaaagggtcacgacgggctgtaccagggactgagcaccgccactaaggatacctacgatgccttgcatatgcaagcactcccaccccgg

SEQ ID NO: 22 - protein, 495 aa, Artificial Sequence
  LTG2065_(LP-M19217-1-CD8 TM-41BB-CD3 zeta)
MLLLVTSLLLCELPHPAFLLIPEVQLVQSGAEVKKPGASVKVSCKASGYTFTSYYMHWVRQAPGQGLEWMGLINPSGGSTSYAQKFQGRVTMTRDTSTSTVYMELSSLRSEDTAVYYCARSDRGITATDAFDIWGQGTMVTVSSGGGGSGGGGSGGGGSQSVLTQPPSVSVAPGRMAKITCGGSDIGNKNVHWYQQKPGQAPVLVVYDDYDRPSGIPERFSGSNSGDAATLTISTVEVGDEADYFCQVWDGSGDPYWMFGGGTQLTVLGAAATTTPAPRPPTPAPTIASQPLSLRPEACRPAAGGAVHTRGLDFACDIYIWAPLAGTCGVLLLSLVITLYCKRGRKKLLYIFKQPFMRPVQTTQEEDGCSCRFPEEEEGGCELRVKFSRSADAPAYQQGQNQLYNELNLGRREEYDVLDKRRGRDPEMGGKPRRKNPQEGLYNELQKDKMAEAYSEIGMKGERRRGKGHDGLYQGLSTATKDTYDALHMQALPPR

SEQ ID NO: 23 - DNA, 1485 bp, Artificial Sequence
  LTG2066 _(LP-M19217-2-CD8 TM-41BB-CD3 zeta)
atgctgctgctggtgaccagcctgctgctgtgcgaactgccgcatccggcgtttctgctgattccggaggtccagctggtacagtctggagctgaggtgaagaagcctggggcctcagtgaaggtctcctgcaaggcttccggatacaccttcaccagctactacatgcactgggtgcgacaggcccctggacaagggtttgagtggatgggattaatcaaccctagtggtagtagcacaagctacgcacagaagttccagggcagagtcaccatgaccagggacacgtccacgagcacagtctacatggagctgagcaacctgagatctgaggacacggccgtgtattactgtgcgagatcggatcggggaattaccgccacggacgcttttgatatctggggccaagggacaatggtcaccgtctcttcaggcggaggaggctccgggggaggaggttccgggggcgggggttcccagtctgtgctgactcagccaccctcggtgccagtggccccagggcagacggccaagattatctgtgggggaagtgacattggaaataaaaatgtccactggtaccagcagaagccaggccaggcccctgtcctggtcgtctatgatgactacgaccggccctcagggatccctgagcgattctctggctccaactctggggacgcggccaccctgacgatcagcacggttgaagtcggggatgaggccgactatttctgtcaggtgtgggacggtagtggtgatccttattgggtgttcggcggagggacccagctcaccgtcttaggtgcggccgcaactaccacccctgcccctcggccgccgactccggccccaaccatcgcaagccaacccctctccttgcgccccgaagcttgccgcccggccgcgggtggagccgtgcatacccgggggctggactttgcctgcgatatctacatttgggccccgctggccggcacttgcggcgtgctcctgctgtcgctggtcatcaccctttactgcaagaggggccggaagaagctgctttacatcttcaagcagccgttcatgcggcccgtgcagacgactcaggaagaggacggatgctcgtgcagattccctgaggaggaagaggggggatgcgaactgcgcgtcaagttctcacggtccgccgacgcccccgcatatcaacagggccagaatcagctctacaacgagctgaacctgggaaggagagaggagtacgacgtgctggacaagcgacgcggacgcgacccggagatgggggggaaaccacggcggaaaaaccctcaggaaggactgtacaacgaactccagaaagacaagatggcggaagcctactcagaaatcgggatgaagggagagcggaggaggggaaagggtcacgacgggctgtaccagggactgagcaccgccactaaggatacctacgatgccttgcatatgcaagcactcccaccccgg

SEQ ID NO: 24 - protein, 495 aa, Artificial Sequence
  LTG2066 _(LP-M19217-2-CD8 TM-41BB-CD3 zeta)
MLLLVTSLLLCELPHPAFLLIPEVQLVQSGAEVKKPGASVKVSCKASGYTFTSYYMHWVRQAPGQGFEWMGLINPSGSSTSYAQKFQGRVTMTRDTSTSTVYMELSNLRSEDTAVYYCARSDRGITATDAFDIWGQGTMVTVSSGGGGSGGGGSGGGGSQSVLTQPPSVPVAPGQTAKIICGGSDIGNKNVHWYQQKPGQAPVLVVYDDYDRPSGIPERFSGSNSGDAATLTISTVEVGDEADYFCQVWDGSGDPYWVFGGGTQLTVLGAAATTTPAPRPPTPAPTIASQPLSLRPEACRPAAGGAVHTRGLDFACDIYIWAPLAGTCGVLLLSLVITLYCKRGRKKLLYIFKQPFMRPVQTTQEEDGCSCRFPEEEEGGCELRVKFSRSADAPAYQQGQNQLYNELNLGRREEYDVLDKRRGRDPEMGGKPRRKNPQEGLYNELQKDKMAEAYSEIGMKGERRRGKGHDGLYQGLSTATKDTYDALHMQALPPR

SEQ ID NO: 25 - DNA, 1485 bp, Artificial Sequence
  LTG2067_(LP-M19217-7-CD8 TM-41BB-CD3 zeta)
atgctgctgctggtgaccagcctgctgctgtgcgaactgccgcatccggcgtttctgctgattccggaggtccagctggtacagtctggagctgaggtgaacaagcctggtgcctcagtgaaggtctcctgcaaggcttctggatacaccttcaccagctactatatgcactgggtgcgacaggcccctggacaagggcttgagtggatgggaatgatcaaccctagtggtggtagcacaagctacgcacagaagttccagggcagagtcaccatgaccagggacacgtccacgagcacagtctacatggagctgagcagcctgagatctgaggacacggccgtgtattactgtgcgagatcggatcggggaattacctccacggacgcttttgatatctggggccaagggacaatggtcaccgtctcttcaggcggaggaggctccgggggaggaggttccgggggcgggggttcccagtctgtgctgactcagccaccctcggtgtcattggccccagggcagacggccaagattacctgtgggggaagtgacattggaaataaaaatgtccactggtaccagcagaagccaggccaggcccctgtcctagtcgtctatgatgattacaaccggccctcagggatccctgagcgattctctggctccaactctggggactcagccaccctgacgatcagcacggtcgaagtcggggatgaggccgactatttctgtcaggtgtgggacggtagtggtgatccttattgggtgttcggcggagggacccagctcaccgttttaggtgcggccgcaactaccacccctgcccctcggccgccgactccggccccaaccatcgcaagccaacccctctccttgcgccccgaagcttgccgcccggccgcgggtggagccgtgcatacccgggggctggactttgcctgcgatatctacatttgggccccgctggccggcacttgcggcgtgctcctgctgtcgctggtcatcaccctttactgcaagaggggccggaagaagctgctttacatcttcaagcagccgttcatgcggcccgtgcagacgactcaggaagaggacggatgctcgtgcagattccctgaggaggaagaggggggatgcgaactgcgcgtcaagttctcacggtccgccgacgcccccgcatatcaacagggccagaatcagctctacaacgagctgaacctgggaaggagagaggagtacgacgtgctggacaagcgacgcggacgcgacccggagatgggggggaaaccacggcggaaaaaccctcaggaaggactgtacaacgaactccagaaagacaagatggcggaagcctactcagaaatcgggatgaagggagagcggaggaggggaaagggtcacgacgggctgtaccagggactgagcaccgccactaaggatacctacgatgccttgcatatgcaagcactcccaccccgg

SEQ ID NO: 26 - protein, 495 aa, Artificial Sequence
  LTG2067 _(LP-M19217-7-CD8 TM-41BB-CD3 zeta)
MLLLVTSLLLCELPHPAFLLIPEVQLVQSGAEVNKPGASVKVSCKASGYTFTSYYMHWVRQAPGQGLEWMGMINPSGGSTSYAQKFQGRVTMTRDTSTSTVYMELSSLRSEDTAVYYCARSDRGITSTDAFDIWGQGTMVTVSSGGGGSGGGGSGGGGSQSVLTQPPSVSLAPGQTAKITCGGSDIGNKNVHWYQQKPGQAPVLVVYDDYNRPSGIPERFSGSNSGDSATLTISTVEVGDEADYFCQVWDGSGDPYWVFGGGTQLTVLGAAATTTPAPRPPTPAPTIASQPLSLRPEACRPAAGGAVHTRGLDFACDIYIWAPLAGTCGVLLLSLVITLYCKRGRKKLLYIFKQPFMRPVQTTQEEDGCSCRFPEEEEGGCELRVKFSRSADAPAYQQGQNQLYNELNLGRREEYDVLDKRRGRDPEMGGKPRRKNPQEGLYNELQKDKMAEAYSEIGMKGERRRGKGHDGLYQGLSTATKDTYDALHMQALPPR

SEQ ID NO: 27 - DNA, 1485 bp, Artificial Sequence
  LTG2068_(LP-M19217-23-CD8 TM-41BB-CD3 zeta)
atgctgctgctggtgaccagcctgctgctgtgcgaactgccgcatccggcgtttctgctgattccggaggtccagctggtacagtctggagctgaggtgaagaagcctggggcctcagtgaaggtctcctgcaaggcatctggatacaccttcaccggctactatatgcactgggtgcggcaggcccctggacaagggcttgagtggataggattaatcaaccctagtggtggtagcacaagctacgaacagaagttccagggcagagtcgccatgaccagggacacgtcaacgagcacagtctacatggagctgagcagcctgagatctgaggacacggccgtgtattactgtgcgagatcggatcggggaattaccgccacggacgcttttgatatctggggccaagggacaatggtcaccgtctcttcaggcggaggaggctccgggggaggaggttccgggggcgggggttcccagtctgtgctgactcagccaccctcggtgtcagtggccccagggcagacggccaagattacctgtgggggaagtgacattggagataaaaatgtccactggtaccagcagaagccaggccaggcccctgtcctggtcgtctatgatgattacgaccggccctcagggatccctgagcgattctctggctccaactctggggacgcggccaccctgacgatcagcacggtcgaagtcggggatgaggccgactatttctgtcaggtgtgggacggtattggtgatccctattgggtgttcggcggagggacccagctcaccgttttaggtgcggccgcaactaccacccctgcccctcggccgccgactccggccccaaccatcgcaagccaacccctctccttgcgccccgaagcttgccgcccggccgcgggtggagccgtgcatacccgggggctggactttgcctgcgatatctacatttgggccccgctggccggcacttgcggcgtgctcctgctgtcgctggtcatcaccctttactgcaagaggggccggaagaagctgctttacatcttcaagcagccgttcatgcggcccgtgcagacgactcaggaagaggacggatgctcgtgcagattccctgaggaggaagaggggggatgcgaactgcgcgtcaagttctcacggtccgccgacgcccccgcatatcaacagggccagaatcagctctacaacgagctgaacctgggaaggagagaggagtacgacgtgctggacaagcgacgcggacgcgacccggagatgggggggaaaccacggcggaaaaaccctcaggaaggactgtacaacgaactccagaaagacaagatggcggaagcctactcagaaatcgggatgaagggagagcggaggaggggaaagggtcacgacgggctgtaccagggactgagcaccgccactaaggatacctacgatgccttgcatatgcaagcactcccaccccgg

SEQ ID NO: 28 - protein, 495 aa, Artificial Sequence
  LTG2068 _(LP-M19217-23-CD8 TM-41BB-CD3 zeta)
MLLLVTSLLLCELPHPAFLLIPEVQLVQSGAEVKKPGASVKVSCKASGYTFTGYYMHWVRQAPGQGLEWIGLINPSGGSTSYEQKFQGRVAMTRDTSTSTVYMELSSLRSEDTAVYYCARSDRGITATDAFDIWGQGTMVTVSSGGGGSGGGGSGGGGSQSVLTQPPSVSVAPGQTAKITCGGSDIGDKNVHWYQQKPGQAPVLVVYDDYDRPSGIPERFSGSNSGDAATLTISTVEVGDEADYFCQVWDGIGDPYWVFGGGTQLTVLGAAATTTPAPRPPTPAPTIASQPLSLRPEACRPAAGGAVHTRGLDFACDIYIWAPLAGTCGVLLLSLVITLYCKRGRKKLLYIFKQPFMRPVQTTQEEDGCSCRFPEEEEGGCELRVKFSRSADAPAYQQGQNQLYNELNLGRREEYDVLDKRRGRDPEMGGKPRRKNPQEGLYNELQKDKMAEAYSEIGMKGERRRGKGHDGLYQGLSTATKDTYDALHMQALPPR

SEQ ID NO: 29 - DNA, 1485 bp, Artificial Sequence
  LTG2069_(LP-M19217-29-CD8 TM-41BB-CD3 zeta)
atgctgctgctggtgaccagcctgctgctgtgcgaactgccgcatccggcgtttctgctgattccggaggtccagctagtacagtctggagctgaggtgaagaagcctggggcctcagtgaaggtctcctgcaaggcttctggatacaccttcaccagctactatatgcactgggtgcgacaggcccctggacaagggcttgagtggatgggaatgatcaaccctagtggtggtagcacaagctacgcacagaagttccagggcagagtcaccatgaccagggacacgtccacgagcacagtctacatggagctgagcagcctgagatctgaggacacggccgtgtattactgtgcgagatcggatcggggaattaccgccacggacgcttttgatatctggggccaagggacaatggtcaccgtctcttcaggcggaggaggctccgggggaggaggttccgggggcgggggttcccagtctgtgctgactcagccaccctcggtgtcagtggccccagggcagacggccaagattacctgtgggggaagtgacattggaaataaaaatgcccactggtaccagcagaagccaggccaggcccctgtcctggtcgtctatgatgattacgaccggccctcagggatctctgagcgattctctggctccaactctggggacgcggccaccctgacgatcagcacggtcgaagtcggggatgaggccgactatttctgtcaggtgtgggacggtagtggtgatcctttttgggtgttcggcggagggacccagctcaccgttttaggtgcggccgcaactaccacccctgcccctcggccgccgactccggccccaaccatcgcaagccaacccctctccttgcgccccgaagcttgccgcccggccgcgggtggagccgtgcatacccgggggctggactttgcctgcgatatctacatttgggccccgctggccggcacttgcggcgtgctcctgctgtcgctggtcatcaccctttactgcaagaggggccggaagaagctgctttacatcttcaagcagccgttcatgcggcccgtgcagacgactcaggaagaggacggatgctcgtgcagattccctgaggaggaagaggggggatgcgaactgcgcgtcaagttctcacggtccgccgacgcccccgcatatcaacagggccagaatcagctctacaacgagctgaacctgggaaggagagaggagtacgacgtgctggacaagcgacgcggacgcgacccggagatgggggggaaaccacggcggaaaaaccctcaggaaggactgtacaacgaactccagaaagacaagatggcggaagcctactcagaaatcgggatgaagggagagcggaggaggggaaagggtcacgacgggctgtaccagggactgagcaccgccactaaggatacctacgatgccttgcatatgcaagcactcccaccccgg

SEQ ID NO: 30 - protein, 495 aa, Artificial Sequence
  LTG2069 _(LP-M19217-29-CD8 TM-41BB-CD3 zeta)
MLLLVTSLLLCELPHPAFLLIPEVQLVQSGAEVKKPGASVKVSCKASGYTFTSYYMHWVRQAPGQGLEWMGMINPSGGSTSYAQKFQGRVTMTRDTSTSTVYMELSSLRSEDTAVYYCARSDRGITATDAFDIWGQGTMVTVSSGGGGSGGGGSGGGGSQSVLTQPPSVSVAPGQTAKITCGGSDIGNKNAHWYQQKPGQAPVLVVYDDYDRPSGISERFSGSNSGDAATLTISTVEVGDEADYFCQVWDGSGDPFWVFGGGTQLTVLGAAATTTPAPRPPTPAPTIASQPLSLRPEACRPAAGGAVHTRGLDFACDIYIWAPLAGTCGVLLLSLVITLYCKRGRKKLLYIFKQPFMRPVQTTQEEDGCSCRFPEEEEGGCELRVKFSRSADAPAYQQGQNQLYNELNLGRREEYDVLDKRRGRDPEMGGKPRRKNPQEGLYNELQKDKMAEAYSEIGMKGERRRGKGHDGLYQGLSTATKDTYDALHMQALPPR

SEQ ID NO: 31 - DNA, 1485 bp, Artificial Sequence
  LTG2070_(LP-M19217-38-CD8 TM-41BB-CD3 zeta)
atgctgctgctggtgaccagcctgctgctgtgcgaactgccgcatccggcgtttctgctgattccggaggtccagctggtacagtctggagctgaggtgaagaggcctggggcctcagtgaaggtctcctgcaaggcttctggatacaccttcaccagctactatatgcactgggtgcgacaggcccctggacgagggcttgagtggatgggattaatcaaccctagtggtggtagcacaagctacgcacaggagttccagggcagagtcaccatgaccagggacatgtccacgagcacagtctacatggagctgagcagcctgagatctgaggacacggccgtgtattactgtgcgagatcggatcggggaattagcgccacggacgcttttgatatctggggccaagggacaatggtcaccgtctcttcaggcggaggaggctccgggggaggaggttccgggggcgggggttcccagtctgtgctgactcagccaccctcggtgtcagtggccccagggcagatggccaagattacctgtgggggaagtgacattggaaataaaaatgtccactggtaccagcagaagccaggccaggcccctgtcctggtcgtctatgatgattacaaccggccctcagggatccctgagcgattctctggctccaactctggggacgcggccaccctgacgatcagcacggtcgaagtcggggatgaggccgactatttctgtcaggtatgggacggtagtggtgatccttattgggtgttcggcggagggacccagctcaccgatttaggtgcggccgcaactaccacccctgcccctcggccgccgactccggccccaaccatcgcaagccaacccctctccttgcgccccgaagcttgccgcccggccgcgggtggagccgtgcatacccgggggctggactttgcctgcgatatctacatttgggccccgctggccggcacttgcggcgtgctcctgctgtcgctggtcatcaccctttactgcaagaggggccggaagaagctgctttacatcttcaagcagccgttcatgcggcccgtgcagacgactcaggaagaggacggatgctcgtgcagattccctgaggaggaagaggggggatgcgaactgcgcgtcaagttctcacggtccgccgacgcccccgcatatcaacagggccagaatcagctctacaacgagctgaacctgggaaggagagaggagtacgacgtgctggacaagcgacgcggacgcgacccggagatgggggggaaaccacggcggaaaaaccctcaggaaggactgtacaacgaactccagaaagacaagatggcggaagcctactcagaaatcgggatgaagggagagcggaggaggggaaagggtcacgacgggctgtaccagggactgagcaccgccactaaggatacctacgatgccttgcatatgcaagcactcccaccccgg

SEQ ID NO: 32 - protein, 495 aa, Artificial Sequence
  LTG2070 _(LP-M19217-38-CD8 TM-41BB-CD3 zeta)
MLLLVTSLLLCELPHPAFLLIPEVQLVQSGAEVKRPGASVKVSCKASGYTFTSYYMHWVRQAPGRGLEWMGLINPSGGSTSYAQEFQGRVTMTRDMSTSTVYMELSSLRSEDTAVYYCARSDRGISATDAFDIWGQGTMVTVSSGGGGSGGGGSGGGGSQSVLTQPPSVSVAPGQMAKITCGGSDIGNKNVHWYQQKPGQAPVLVVYDDYNRPSGIPERFSGSNSGDAATLTISTVEVGDEADYFCQVWDGSGDPYWVFGGGTQLTDLGAAATTTPAPRPPTPAPTIASQPLSLRPEACRPAAGGAVHTRGLDFACDIYIWAPLAGTCGVLLLSLVITLYCKRGRKKLLYIFKQPFMRPVQTTQEEDGCSCRFPEEEEGGCELRVKFSRSADAPAYQQGQNQLYNELNLGRREEYDVLDKRRGRDPEMGGKPRRKNPQEGLYNELQKDKMAEAYSEIGMKGERRRGKGHDGLYQGLSTATKDTYDALHMQALPPR

SEQ ID NO: 33 - DNA, 1485 bp, Artificial Sequence
  LTG2071_(LP-M19217-40-CD8 TM-41BB-CD3 zeta)
atgctgctgctggtgaccagcctgctgctgtgcgaactgccgcatccggcgtttctgctgattccggaggtccagctggtacagtctggagctgaggtgaagaggcctggggcctcagtgaaggtctcctgcaaggcttctggatacaccttcaccagctactatatgcactgggtgcgacaggcccctggacaagggcttgtgtggatgggattaatcaaccctagtggtggcagcacaagctacgcacagaagttccagggcagagtcaccatgaccagggacacgtccacgagcacagtctacatggagctgagcagcctgagatctgaggacacggccgtgtattactgtgcgagatcggatcggggaattaccgccacggacgcttttgatatctggggccaagggacaatggtcaccgtctcttcaggcggaggaggctccgggggaggaggttccgggggcgggggttcccagtctgtgctgactcagccaccctcggtctcagtggccccagggcagacggccaagactacctgtgggggaagtgacattggaaataaaaatgtccactggtaccagcagaagccaggccaggcccctgtcctggtcgtctatgatgattacgaccggccctcagggatccctgagcgattctctggctccaactctggggacgcggccaccctgacgatcagcacggtcgaagtcggggatgaggccgactatgtctgtcaggtgtgggacggtagtggtgatccttattgggtgttcggcggagggacccagctcaccgttttaggtgcggccgcaactaccacccctgcccctcggccgccgactccggccccaaccatcgcaagccaacccctctccttgcgccccgaagcttgccgcccggccgcgggtggagccgtgcatacccgggggctggactttgcctgcgatatctacatttgggccccgctggccggcacttgcggcgtgctcctgctgtcgctggtcatcaccctttactgcaagaggggccggaagaagctgctttacatcttcaagcagccgttcatgcggcccgtgcagacgactcaggaagaggacggatgctcgtgcagattccctgaggaggaagaggggggatgcgaactgcgcgtcaagttctcacggtccgccgacgcccccgcatatcaacagggccagaatcagctctacaacgagctgaacctgggaaggagagaggagtacgacgtgctggacaagcgacgcggacgcgacccggagatgggggggaaaccacggcggaaaaaccctcaggaaggactgtacaacgaactccagaaagacaagatggcggaagcctactcagaaatcgggatgaagggagagcggaggaggggaaagggtcacgacgggctgtaccagggactgagcaccgccactaaggatacctacgatgccttgcatatgcaagcactcccaccccgg

SEQ ID NO: 34 - protein, 495 aa, Artificial Sequence
  LTG2071 _(LP-M19217-40-CD8 TM-41BB-CD3 zeta)
MLLLVTSLLLCELPHPAFLLIPEVQLVQSGAEVKRPGASVKVSCKASGYTFTSYYMHWVRQAPGQGLVWMGLINPSGGSTSYAQKFQGRVTMTRDTSTSTVYMELSSLRSEDTAVYYCARSDRGITATDAFDIWGQGTMVTVSSGGGGSGGGGSGGGGSQSVLTQPPSVSVAPGQTAKTTCGGSDIGNKNVHWYQQKPGQAPVLVVYDDYDRPSGIPERFSGSNSGDAATLTISTVEVGDEADYVCQVWDGSGDPYWVFGGGTQLTVLGAAATTTPAPRPPTPAPTIASQPLSLRPEACRPAAGGAVHTRGLDFACDIYIWAPLAGTCGVLLLSLVITLYCKRGRKKLLYIFKQPFMRPVQTTQEEDGCSCRFPEEEEGGCELRVKFSRSADAPAYQQGQNQLYNELNLGRREEYDVLDKRRGRDPEMGGKPRRKNPQEGLYNELQKDKMAEAYSEIGMKGERRRGKGHDGLYQGLSTATKDTYDALHMQALPPR

SEQ ID NO: 35 - DNA, 66 bp, Artificial Sequence
  DNA CD8 transmembrane domain
atttgggccccgctggccggcacttgcggcgtgctcctgctgtcgctggtcatcaccctttactgc

SEQ ID NO: 36 - protein, 22 aa, Artificial Sequence
  CD8 transmembrane domain
IWAPLAGTCGVLLLSLVITLYC

SEQ ID NO: 37 - DNA, 141 bp, Artificial Sequence
  DNA CD8 hinge domain
actaccacccctgcccctcggccgccgactccggccccaaccatcgcaagccaacccctctccttgcgccccgaagcttgccgcccggccgcgggtggagccgtgcatacccgggggctggactttgcctgcgatatctac

SEQ ID NO: 38 - protein, 46 aa, Artificial Sequence
  CD8 hinge domain
TTTPAPRPPTPAPTIASQPLSLRPEACRPAAGGAVHTRGLDFACDI

SEQ ID NO: 39 - protein, 69 aa, Artificial Sequence
  hinge and  transmembrane region of CD8.alpha. (NCBI RefSeq: NP.sub.--001759.3)
TTTPAPRPPTPAPTIASQPLSLRPEACRPAAGGAVHTRGLDFACDIYIWAPLAGTCGVLLLSLVITLYC

SEQ ID NO: 40 - DNA, 126 bp, Artificial Sequence
  signaling domain of 4-1BB
aagaggggccggaagaagctgctttacatcttcaagcagccgttcatgcggcccgtgcagacgactcaggaagaggacggatgctcgtgcagattccctgaggaggaagaggggggatgcgaactg

SEQ ID NO: 41 - protein, 42 aa, Artificial Sequence
  signaling domain of 4-1BB
KRGRKKLLYIFKQPFMRPVQTTQEEDGCSCRFPEEEEGGCEL

SEQ ID NO: 42 - DNA, 336 bp, Artificial Sequence
  intracellular signaling domain of CD3-zeta
cgcgtcaagttctcacggtccgccgacgcccccgcatatcaacagggccagaatcagctctacaacgagctgaacctgggaaggagagaggagtacgacgtgctggacaagcgacgcggacgcgacccggagatgggggggaaaccacggcggaaaaaccctcaggaaggactgtacaacgaactccagaaagacaagatggcggaagcctactcagaaatcgggatgaagggagagcggaggaggggaaagggtcacgacgggctgtaccagggactgagcaccgccactaaggatacctacgatgccttgcatatgcaagcactcccaccccgg

SEQ ID NO: 43 - protein, 112 aa, Artificial Sequence
  CD3-zeta
RVKFSRSADAPAYQQGQNQLYNELNLGRREEYDVLDKRRGRDPEMGGKPRRKNPQEGLYNELQKDKMAEAYSEIGMKGERRRGKGHDGLYQGLSTATKDTYDALHMQALPPR

SEQ ID NO: 44 - DNA, 336 bp, Artificial Sequence
  intracellular signaling domain of CD3-zeta, variant
cgcgtcaagttctcacggtccgccgacgcccccgcatataaacagggccagaatcagctctacaacgagctgaacctgggaaggagagaggagtacgacgtgctggacaagcgacgcggacgcgacccggagatgggggggaaaccacggcggaaaaaccctcaggaaggactgtacaacgaactccagaaagacaagatggcggaagcctactcagaaatcgggatgaagggagagcggaggaggggaaagggtcacgacgggctgtaccagggactgagcaccgccactaaggatacctacgatgccttgcatatgcaagcactcccaccccgg

SEQ ID NO: 45 - protein, 112 aa, Artificial Sequence
  CD3-zeta signaling domain, variant
RVKFSRSADAPAYKQGQNQLYNELNLGRREEYDVLDKRRGRDPEMGGKPRRKNPQEGLYNELQKDKMAEAYSEIGMKGERRRGKGHDGLYQGLSTATKDTYDALHMQALPPR

SEQ ID NO: 46 - DNA, 726 bp, Artificial Sequence
  ScFv CD19 (FMC63)
gacattcagatgactcagaccacctcttccttgtccgcgtcactgggagacagagtgaccatctcgtgtcgcgcaagccaggatatctccaagtacctgaactggtaccaacagaagcccgacgggactgtgaagctgctgatctaccacacctcacgcctgcacagcggagtgccaagcagattctccggctccggctcgggaaccgattactcgcttaccattagcaacctcgagcaggaggacatcgctacctacttctgccagcaaggaaataccctgccctacaccttcggcggaggaaccaaattggaaatcaccggcggaggaggctccgggggaggaggttccgggggcgggggttccgaagtgaagctccaggagtccggccccggcctggtggcgccgtcgcaatcactctctgtgacctgtaccgtgtcgggagtgtccctgcctgattacggcgtgagctggattcggcagccgccgcggaagggcctggaatggctgggtgtcatctggggatccgagactacctactacaactcggccctgaagtcccgcctgactatcatcaaagacaactcgaagtcccaggtctttctgaagatgaactccctgcaaactgacgacaccgccatctattactgtgctaagcactactactacggtggaagctatgctatggactactgggggcaaggcacttcggtgactgtgtcaagc

SEQ ID NO: 47 - protein, 242 aa, Artificial Sequence
  ScFv CD19 (FMC63)
DIQMTQTTSSLSASLGDRVTISCRASQDISKYLNWYQQKPDGTVKLLIYHTSRLHSGVPSRFSGSGSGTDYSLTISNLEQEDIATYFCQQGNTLPYTFGGGTKLEITGGGGSGGGGSGGGGSEVKLQESGPGLVAPSQSLSVTCTVSGVSLPDYGVSWIRQPPRKGLEWLGVIWGSETTYYNSALKSRLTIIKDNSKSQVFLKMNSLQTDDTAIYYCAKHYYYGGSYAMDYWGQGTSVTVSS

SEQ ID NO: 48 - DNA, 747 bp, Artificial Sequence
  anti-CD33 ScFv (LTG1936)
caggtgcagctggtgcaatctggggcagaggtgaaaaagcccggggagtctctgaggatctcctgtaagggttctggattcagttttcccacctactggatcggctgggtgcgccagatgcccgggaaaggcctggagtggatggggatcatctatcctggtgactctgataccagatacagcccgtccttccaaggccaggtcaccatctcagccgacaagtccatcagcaccgcctacctgcagtggagcagcctgaaggcctcggacaccgccatgtattactgtgcgagactagttggagatggctacaatacgggggcttttgatatctggggccaagggacaatggtcaccgtctcttcaggaggtggcgggtctggtggtggcggtagcggtggtggcggatccgatattgtgatgacccacactccactctctctgtccgtcacccctggacagccggcctccatctcctgcaagtctagtcagagcctcctgcatagtaatggaaagacctatttgtattggtacctgcagaagccaggccagcctccacagctcctgatctatggagcttccaaccggttctctggagtgccagacaggttcagtggcagcgggtcagggacagatttcacactgaaaatcagccgggtggaggctgaggatgttggggtttattactgcatgcaaagtatacagcttcctatcaccttcggccaagggacacgactggagattaaa

SEQ ID NO: 49 - protein, 249 aa, Artificial Sequence
  anti-CD33 ScFv (LTG1936)
QVQLVQSGAEVKKPGESLRISCKGSGFSFPTYWIGWVRQMPGKGLEWMGIIYPGDSDTRYSPSFQGQVTISADKSISTAYLQWSSLKASDTAMYYCARLVGDGYNTGAFDIWGQGTMVTVSSGGGGSGGGGSGGGGSDIVMTHTPLSLSVTPGQPASISCKSSQSLLHSNGKTYLYWYLQKPGQPPQLLIYGASNRFSGVPDRFSGSGSGTDFTLKISRVEAEDVGVYYCMQSIQLPITFGQGTRLEIK

SEQ ID NO: 50 - DNA, 732 bp, Artificial Sequence
  anti-mesothelin ScFv (LTG1904)
gaggtccagctggtacagtctgggggaggcttggtacagcctggggggtccctgagactctcctgtgcagcctctggattcacctttgatgattatgccatgcactgggtccggcaagctccagggaagggcctggagtgggtctcaggtattagttggaatagtggtagcataggctatgcggactctgtgaagggccgattcaccatctccagagacaacgccaagaactccctgtatctgcaaatgaacagtctgagagctgaggacacggccttgtattactgtgcaaaagatttatcgtcagtggctggaccctttaactactggggccagggcaccctggtcaccgtctcctcaggaggtggcgggtctggtggaggcggtagcggcggtggcggatcctcttctgagctgactcaggaccctgctgtgtctgtggccttgggacagacagtcaggatcacatgccaaggagacagcctcagaagctattatgcaagctggtaccagcagaagccaggacaggcccctgtacttgtcatctatggtaaaaacaaccggccctcagggatcccagaccgattctctggctccagctcaggaaacacagcttccttgaccatcactggggctcaggcggaggatgaggctgactattactgtaactcccgggacagcagtggtaaccatctggtattcggcggaggcacccagctgaccgtcctcggt

SEQ ID NO: 51 - protein, 244 aa, Artificial Sequence
  anti-mesothelin ScFv (LTG1904)
EVQLVQSGGGLVQPGGSLRLSCAASGFTFDDYAMHWVRQAPGKGLEWVSGISWNSGSIGYADSVKGRFTISRDNAKNSLYLQMNSLRAEDTALYYCAKDLSSVAGPFNYWGQGTLVTVSSGGGGSGGGGSGGGGSSSELTQDPAVSVALGQTVRITCQGDSLRSYYASWYQQKPGQAPVLVIYGKNNRPSGIPDRFSGSSSGNTASLTITGAQAEDEADYYCNSRDSSGNHLVFGGGTQLTVLG